European Patent Application EP 4 155 410 A1, published March 29, 2023. Title: NUCLEIC ACID CONSTRUCT, RECOMBINANT INFLUENZA VIRUS, METHOD FOR PREPARING A RECOMBINANT INFLUENZA VIRUS, COMPOSITION AND USE. Applicant: FUNDAÇÃO OSWALDO CRUZ. Application BR PCT/BR2021/050216, filed May 20, 2021. The sequence listing filed with the application follows.

SEQUENCE LISTING (9 sequences)

SEQ ID NO: 1 - DNA, 3147 bp, synthetic construct
  misc_feature 1..3147: note = Plasmid pPRNA166x178
  source 1..3147: mol_type = other DNA
agcaaaagcaggagtttaactaaatccaaaccagaaaataataaccattggatcgatctgtctagtagtcggaataattagcctaatattgcaaataggaaatataatctcaatctagattagccattcaattcaaaccggaaatcaaaaccatactggaatctactctagactcgagagctagcgtcgactgcttctgggttgaattaatcagggggctacctgaggaggacgcaatctggactagtgggagcatcatttctttttgtggtgtgaatggtgatactgtagattggtcttggccagacggtgctgagttgccgttcaccattgacaagtagtttgttcaaaaaactccttgtttctactaataacccggcggcccaaaatgccgactcggagcgaaagatatacctcccccggggccgggaggtcgcgtcaccgaccacgccgccggcccaggcgacgcgcgacacggacacctgtccccaaaaacgccaccatcgcagccacacacggagcgcccggggccctctctggtcaaccccaggacacacgcgggagcagcgccgggccggacgccctcccggccgcccgtgccacacgcaggggccggcccgtaagcttggcgtaatcatggtcatagctgtttcctgtgtgaaattgttatccgctcacaattccacacaacatacgagccggaagcataaagtgtaaagcctggggtgcctaatgagtgagctaactcacattaattgcgttgcgctcactgcccgctttccagtcgggaaacctgtcgtgccagctgcattaatgaatcggccaacgcgcggggagaggcggtttgcgtattgggcgctcttccgcttcctcgctcactgactcgctgcgctcggtcgttcggctgcggcgagcggtatcagctcactcaaaggcggtaatacggttatccacagaatcaggggataacgcaggaaagaacatgtgagcaaaaggccagcaaaaggccaggaaccgtaaaaaggccgcgttgctggcgtttttccataggctccgcccccctgacgagcatcacaaaatcgacgctcaagtcagaggtggcgaaacccgacaggactataaagataccaggcgtttccccctggaagctccctcgtgcgctctctcctgttccgaccctgccgcttaccggatacctgtccgcctttttcccttcgggaagcgtggcgctttctcatagctcacgctgtaggtatctcagttcggtgtaggtcgttcgctccaagctgggctgtgtgcacgaaccccccgttcagcccgaccgctgcgccttatccggtaactatcgtcttgagtccaacccggtaagacacgacttatcgccactggcagcagccactggtaacaggattagcagagcgaggtatgtaggcggtgctacagagttcttgaagtggtggcctaactacggctacactagaaggacagtatttggtatctgcgctctctgctgaagccagttaccttcggaaaaagagagttggtagctcttgatccggcaaacaaaccaccgctggtagcggtggtttttttgtttgcaagcagcagattacgcgcagaaaaaaaggatctcaagaagatcctttgatcttttctacggggtctgacgctcagtggaacgaaaactcacgttaagggattttggtcatgagattatcaaaaaggatcttcacctagatccttttaaattaaaatgaagttttaaatcaatctaaagtatatatgagtaaacttggtctgacagttaccaatgcttaatcagtgaggcacctatctcagcgatctgtctatttcgttcatccatagttgcctgactccccgtcgtgtagataactacgatacgggagggcttaccatctggccccagtgctgcaatgataccgcgagacccacgctcaccggctccagatttatcagcaataaaccagccagccggaagggccgagcgcagaagtggtcctgcaactttatccgcctccatccagtctattaattgttgccgggaagctagagtaagtagttcgccagttaatagtttgcgcaacgttgttgccattgctacaggcatcgtggtgtcacgctcgtcgtttggtatggcttcattcagctccggttcccaacgatcaaggcgagttacatgatcccccatgttgtgcaaaaagcggttagctccttcggtcctccgatcgttgtcagaagtaagttggccgcagtgttatcactcatggttatggcagcactgcataattctcttactgtcatgccatccgtaagatgcttttctgtgactggtgagtactcaaccaagtcattctgagaatagtgtatgcggcgaccgagttgctcttgcccggcgtcaatacgggataataccgcgccacatagcagaactttaaaagtgctcatcattggaaaacgttcttcggggcgaaaactctcaaggatcttaccgctgttgagatccagttcgatgtaacccactcgtgcacccaactgatcttcagcatcttttactttcaccagcgtttctgggtgagcaaaaacaggaaggcaaaatgccgcaaaaaagggaataagggcgacacggaaatgttgaatactcatactcttcctttttcaatatattattgaagcatttatcagggttattgtctcatgagcggatacatatttgaatgtatttagaaaaataaacaaataggggttccgcgcacatttccccgaaaagtgccacctgacgtctaagaaaccattattatcatgacattaacctataaaaataggcgtatcacgaggccctttcgtctcgcgcgtttcggtgatgacggtgaaaacctctgacacatgcagctcccggagacggtcacagcttgtctgtaagcggatgccgggagcagacaagcccgtcagggcgcgtcagcgggtgttggcgggtgtcggggctggcttaactatgcggcatcagagcagattgtactgagagtgcaccatatgcggtgtgaaataccgcacagatgcgtaaggagaaaataccgcatcaggcgccattcgccattcaggctgcgcaactgttgggaagggcgatcg

SEQ ID NO: 2 - DNA, 540 bp, Homo sapiens
  source 1..540: mol_type = other DNA
atgttccatgtttcttttaggtatatctttggacttcctcccctgatccttgttctgttgccagtagcatcatctgattgtgatattgaaggtaaagatggcaaacaatatgagagtgttctaatggtcagcatcgatcaattattggacagcatgaaagaaattggtagcaattgcctgaataatgaatttaacttttttaaaagacatatctgtgatgctaataaggaaggtatgtttttattccgtgctgctcgcaagttgaggcaatttcttaaaatgaatagcactggtgattttgatctctccacttattaaaagtttcagaaggcacaacaatactgttgaactgcactggccaggttaaaggaagaaaaccagctgccctgggtgaagcccaaccaacaaagagagtttggaagaaaataaatctttaaaggaacagaaaaaactgaatgacttgtgtttcctaaagagactattacaagagagataaaaacttgttggaataaaattttgatgggcactaaagaacactga

SEQ ID NO: 3 - DNA, 529 bp, Sus scrofa
  source 1..529: mol_type = other DNA
atgttccatgtttcttttaggtatatcttcggaattcctcccctgatccttgttctgttgccagtagcatcatctgattgtgatattgaaggtaaagacggcggagtgtatcagaatgttctaatggtcagcatcgatgacttggacaggatgatagactttgatagcaattgcctgaataacgaacctaactttttaaaaaaacattcatgtgatgataataaggaagcttcatttttatatcgtgctgctcgaaagttgaagcaatttattaaaatgaatatcagtgaggagttcaatcaccatctatcaacagtttcacagggcacattaacactgttcaactgcaccagcaaggttaaaggaagaaaaccaccttccctgggtgaagcccaactcactaagaacttggaagaaaataaatctttaaaggaacagaaaagacagggggacttgtgtttcctaaagatactactacagaagataaaacttgttggaataaaattttgaggggtgctaaagaatattg

SEQ ID NO: 4 - DNA, 464 bp, Mus musculus
  source 1..464: mol_type = other DNA
atgttccatgtttcttttagatatatctttggaattcctccactgatccttgttctgctgcctgtcacatcatctgagtgccacattaaagacaaagaaggtaaagcatatgagagtgtactgatgatcagcatcgatgaattggacaaaatgacaggaactgatagtaattgcccgaataatgaaccaaacttttttagaaaacatgtatgtgatgatacaaaggaagctgcttttctaaatcgtgctgctcgcaagttgaagcaatttcttaaaatgaatatcagtgaagaattcaatgtccacttactaacagtatcacaaggcacacaaacactggtgaactgcacaagtaaggaagaaaaaaacgtaaaggaacagaaaaagaatgatgcatgtttcctaaagagactactgagagaaataaaacttgttggaataaaattttgaagggcagtatataa

SEQ ID NO: 5 - protein, 175 aa, Homo sapiens
MFHVSFRYIFGLPPLILVLPVASSSDCDIEGKDGKQYESVLMVSIDQLLDSMKEIGSNCLNEFNFFKRHICDANKEGMFLFRAARKLRQFLKMNSTGDFDLHLKVSEGTTILLNCTGQVKGRKPAALGEAQPTKSLEENKSLKEQKKLNDLCFLKRLLQEIKTCWNKILMGTKEH

SEQ ID NO: 6 - protein, 152 aa, Mus musculus
MFHVSFRYIFGIPPPLILVLPVTSSECHIKDKEGKAYESVLMISIDELDKMTGTDSNCPNNEPNFFRKHVCDTKEAAFLNRAARKLKQFLKMNISEEFNVHLTVSQGTQTLVNCTSKEQKNVKEQKKNDACFLKRLLREIKTCWNKILKGSI

SEQ ID NO: 7 - protein, 176 aa, Sus scrofa
MFHVSFRYIFGIPPPLILVLPVASSSDCDIEGKDGGVYQNVLMVSIDDLDRMIDFDSNCLNNEPNFLKKHSCDDNKEASFLYRAARKLKQFIKMNISEEFNHHLSTVSQGTLTLFNCTSKVKGRKPSLGEAQLTKNLEENKSLKEQKRQGDLCFLKILLQKIKTCWNKILRGAKEY

SEQ ID NO: 8 - DNA, 469 bp, Mus musculus
  source 1..469: mol_type = other DNA
atgttccacgtgtcttttagatacatttttgggattccacctctgattctggtcctgctgcctgtcacctcctctctgagtgtcatattaaggacaaagagagggcaaagcttacgaaagcgtgctgatgatctccattgacgagctggataagatgaccggaacagattctaactgccccaacaatgagcctaatttctttcggaaacgtctgtgacgataccaaggaagccgctttcctgaacagggcagccagaaagctgaaacagttcctgaagatgaacatctctgaggagttcaacgtgcatctgctgacagtcagtcagggcactcagaccctggtgaattgcactagcaaggaggagaagaacgtgaaggaacagaagaaaaatgacgcctgttttctgaagagaggctgctgcgggaaatcaagacctgctggaacaaaatcctgaaaggctcaatctga

SEQ ID NO: 9 - DNA, 3835 bp, synthetic construct
  misc_feature 1..3835: note = Plasmid pPRNA166-IL7-178
  source 1..3835: mol_type = other DNA
agcaaaagcaggagtttaactaaatccaaaccagaaaataataaccattggatcgatctgtctagtagtcggaataattagcctaatattgcaaataggaaatataatctcaatctagattagccattcaattcaaaccggaaatcaaaaccatactggaatctactctagactcgagcgcgccaccatgttccacgtgtcttttagatacatttttgggattccacctctgattctggtcctgctgcctgtcacctcctctgagtgtcatattaaggacaaagagggcaaagcttacgaaagcgtgctgatgatctccattgacgagctggataagatgaccggaacagattctaactgccccaacaatgagcctaatttctttcggaaacacgtctgtgacgataccaaggaagccgctttcctgaacagggcagccagaaagctgaaacagttcctgaagatgaacatctctgaggagttcaacgtgcatctgctgacagtcagtcagggcactcagaccctggtgaattgcactagcaaggaggagaagaacgtgaaggaacagaagaaaatgacgcctgttttctgaagaggctgctgcgggaaatcaagacctgctggaacaacaaaatcctgaaaggctcaatctgagctagcgtcgactgcttctgggttgaattaatcagggggctacctgaggaggacgcaatctggactagtgggagcatcatttctttttgtggtgtgaatggtgatactgtagattggtcttggccagacggtgctgagttgccgttcaccattgacaagtagtttgttcaaaaaaactccttgtttctactaataacccggcggcccaaaatgccgactcggagcgaaagatatacctcccccggggccgggaggtcgcgtcaccgaccacgccgccggcccaggcgacgcgcgacacggacacctgtccccaaaaacgccaccatcgcagccacacacacggagcgcccggggccctctctggtcaaccccaggacacacgcgggagcagcgccgggccggggacgccctcccggccgcccgtgccacacgcaggggccggcccgtaagcttggcgtaatcatggtcatagctgtttcctgtgtgaaattgttatccgctcacaattccacacaacatacgagccggaagcataaagtgtaaagcctggggtgcctaatgagtgagctaactcacattaattgcgttgcgctcactgcccgctttccagtcgggaaacctgtcgtgccagctgcattaatgaatcggccaacgcgcggggagaggcggtttgcgtattgggcgctctcttccgcttcctcgctcactgactcgctgcgctcggtcgttcggctgcggcgagcggtatcagctcactcaaaggcggtaatacggttatccacagaatcaggggataacgcaggaaagaacatgtgagcaaaaggccagcaaaaggccaggaaccgtaaaaggccgcgttgctggcgtttttccataggctccgcccccctgacgagcatcacaaaaatcgacgctcaagtcagaggtggcgaaacccgacaggactataaagataccaggcgtttccccctggaagctccctcgtgcgctctcctgttccgaccctgccgcttaccggatacctgtccgcctttctcccttcgggaagcgtggcgctttctcatagctcacgctgtaggtatctcagttcggtgtaggtcgttcgctccaagctgggctgtgtgcacgaaccccccgttcagcccgaccgctgcgccttatccggtaactatcgtcttgagtccaacccggtaagacacgacttatcgccactggcagcagccactggtaacaggattagcagagcgaggtatgtaggcggtgctacagagttcttgaagtggtggcctaactacggctacactagaaggacagtatttggtatctgcgctctgctgaagccagttaccttcggaaaaagagttggtagctcttgatccggcaaacaaaccaccaccgctggtagcggtggtttttttgtttgcaagcagcagattacgcgcagaaaaaaaggatctcaagaagatcctttgatcttttctacggggtctgacgctcagtggaacgaaaactcacgttaagggattttggtcatgagattatcaaaaaggatcttcacctagatccttttaaattaaaaatgaagttttaaatcaatctaaagtatatatgagtaaacttggtctgacagttaccaatgcttaatcagtgaggcacctatctcagcgatctgtctatttcgttcatccatagttgcctgactccccgtcgtgtagataactacgatacgggagggcttaccatctggccccagtgctgcaatgataccgcgagacccacgctcaccggctccagatttatcagcaataaaccagccagccggaagggccgagcgcagaagtggtcctgcaactttatccgcctccatccagtctattaattgttgccgggaagctagagtaagtagttcgccagttaatagtttgcgcaacgttgttgccattgctacaggcatcgtggtgtcacgctcgtcgtttggtatggcttcattcagctccggttcccaacgatcaaggcgagttacatgatcccccatgttgtgcaaaaagcggttagctccttcggtcctccgatcgttgtcagaagtaagttggccgcagtgttatcactcatggttatggcagcactgcataattctcttactgtcatgccatccgtaagatgcttttctgtgactggtgagtactcaaccaagtcattctgagaatagtgtatgcggcgaccgagttgctcttgcccggcgtcaatacgggataataccgcgccacatagcagaactttaaaagtgctcatcattggaaaacgttcttcggggcgaaaactctctcaaggatcttaccgctgttgagatccagttcgatgtaacccactcgtgcacccaactgatcttcagcatcttttactttcaccagcgtttctgggtgagcaaaaacaggaaggcaaaatgccgcaaaaagggaataagggcgacacggaaatgttgaatactcatactcttcctttttcaatattattgaagcatttatcagggttttgtctcatgagcggatacatatttgaatgtatttagaaaaataaacaaataggggttccgcgcacatttccccgaaaagtgccacctgacgtctaagaaaccattattatcatgacattaacctataaaaataggcgtatcacgaggccctttcgtctcgcgcgtttcggtgatgacggtgaaaacctctgacacatgcagctcccggagacggtcacagcttgtctgtaagcggatgccgggagcagacaagcccgtcagggcgcgtcagcgggtgttggcgggtgtcggggctggcttaactatgcggcatcagagcagattgtactgagagtgcaccatatgcggtgtgaaataccgcacagatgcgtaaggagaaaataccgcatcaggcgccattcgccattcaggctgcgcaactgttgggaagggcgatcggtgcgggcctcttcgctattacgccagctggcgaaagggggatgtgctgcaaggcgattaagttgggtaacgccagggttttcccagtcacgacgttgtaaaacgacggccagtgaattcgagctcgtcccattcgccattaccgaggggacggtcccctcggaatgttgcccagccggcgccagcgaggaggctgggaccatgccggcc